European Patent Application EP 4 393 958 A1, published July 3, 2024. Title: LONG-ACTING RECOMBINANT HUMAN INTERLEUKIN-2 FUSION PROTEIN, AND PREPARATION METHOD THEREFOR AND APPLICATION THEREOF. Applicant: Beijing VDJBIO Co., Ltd. The sequence listing filed with the application follows.

SEQUENCE LISTING (5 sequences)

SEQ ID NO: 1 - protein, 133 aa, Artificial Sequence
APTSSSTKKTQLQLEHLLLDLQMILNGINNYKNPKLTRMLTFKFYMPKKATELKHLQCLEEELKPLEEVLNLAQSKNFHLRPRDLISNINVIVLELKGSETTFMCEYADETATIVEFLNRWITFAQSIISTLT

SEQ ID NO: 2 - protein, 585 aa, Artificial Sequence [sequence omitted]

SEQ ID NO: 3 - DNA, 2187 bp, Artificial Sequence
gcaccaactagcagcagcactaagaagacccagctgcaactcgaacatctgctgctcgacctgcaaatgatcctgaatgggattaacaactataagaatcccaagctcactcggatgctcaccttcaagttctacatgcccaagaaagctactgaactcaaacatctgcaatgtctcgaagaggaactgaagccactggaagaggtgctgaatctggcccaatctaagaatttccacctgaggcctagggatctgataagcaatatcaacgtgattgtgctggagctgaagggttctgaaacaacctttatgtgtgagtacgcagacgaaaccgccaccatcgtcgagttcctcaatcggtggatcaccttcgctcagagcatcatctccacactcacaggaggcggtgggagtggtggtggagggtcagacgctcacaagagcgaggtggctcatcggttcaaagacctcggcgaggagaacttcaaggccctggtcctgatcgcctttgcccagtacctgcaacagtgtccctttgaagatcatgtcaagctcgtcaacgaggtgactgagttcgccaagacatgcgtcgcagacgagagtgccgagaattgcgacaaatccctccacaccctgtttggcgataagctctgtactgtcgctactctgagggagacatacggcgagatggctgactgctgcgccaagcaggagcccgagcggaatgaatgctttctgcaacacaaagacgacaatcctaatctgccaaggctcgtcagaccagaggtggatgtgatgtgtaccgcctttcatgataatgaggaaacctttctcaagaagtatctgtatgaaattgctagaaggcacccatacttctatgctcctgagctgctgttcttcgccaaacgctacaaggctgctttcactgaatgctgccaggcagccgacaaagcagcctgcctcctgccaaagctcgacgaactccgggacgaagggaaggcctcaagtgccaagcagagactgaagtgcgcaagcctccagaaattcggagaaagggcattcaaggcttgggcagtggcaaggctgtcccagaggtttcctaaggccgaatttgccgaagtctctaaactggtcacagacctgaccaaagtgcataccgaatgttgccacggcgacctcctggagtgcgctgacgatagggcagacctggccaaatacatttgcgagaaccaggatagtataagtagcaaactcaaggagtgctgtgagaagcctctcctggagaagtcccactgcatcgccgaagtggagaacgatgagatgccagctgacctccctagcctggcagccgactttgtcgaatcaaaggacgtctgcaagaattacgccgaggcaaaggatgtgttcctgggaatgtttctgtacgagtatgccagaaggcaccctgactattcagtcgtgctgctgctgcgcctggccaagacttatgaaactaccctggagaagtgttgcgcagctgccgacccacacgagtgttatgccaaggtgttcgatgagttcaagccactcgtcgaggagcctcagaacctgatcaagcagaactgcgaactcttcgagcagctgggagagtacaaattccagaacgccctgctggtgcggtacaccaagaaggtgccacaggtgtctacacctacactggttgaagtgtccagaaacctcggcaaggtgggaagcaaatgctgcaaacatcccgaggcaaagcggatgccatgcgcagaagattacctctctgtggtgctcaatcaactgtgcgtgctgcacgagaagacccccgtcagtgacagagtgaccaaatgctgcactgagagtctggtcaatagacggccatgcttcagtgccctggaggtggacgaaacatacgttcccaaagagttcaacgccgaaactttcacctttcatgctgacatttgtaccctgtcagagaaggagcggcagattaagaaacaaactgccctggtggaactggtgaaacacaagcctaaggcaaccaaagaacaactgaaggccgtcatggacgatttcgctgccttcgtcgagaagtgttgtaaggctgacgacaaggagacatgtttcgccgaagagggcaagaaactggttgctgccagccaagctgcactgggactgtga

SEQ ID NO: 4 - protein, 728 aa, Artificial Sequence
APTSSSTKKTQLQLEHLLLDLQMILNGINNYKNPKLTRMLTFKFYMPKKATELKHLQCLEEELKPLEEVLNLAQSKNFHLRPRDLISNINVIVLELKGSETTFMCEYADETATIVEFLNRWITFAQSIISTLTGGGGSGGGGSDAHKSEVAHRFKDLGEENFKALVLIAFAQYLQQCPFEDHVKLVNEVTEFAKTCVADESAENCDKSLHTLFGDKLCTVATLRETYGEMADCCAKQEPERNECFLQHKDDNPNLPRLVRPEVDVMCTAFHDNEETFLKKYLYEIARRHPYFYAPELLFFAKRYKAAFTECCQAADKAACLLPKLDELRDEGKASSAKQRLKCASLQKFGERAFKAWAVARLSQRFPKAEFAEVSKLVTDLTKVHTECCHGDLLECADDRADLAKYICENQDSISSKLKECCEKPLLEKSHCIAEVENDEMPADLPSLAADFVESKDVCKNYAEAKDVFLGMFLYEYARRHPDYSVVLLLRLAKTYETTLEKCCAAADPHECYAKVFDEFKPLVEEPQNLIKQNCELFEQLGEYKFQNALLVRYTKKVPQVSTPTLVEVSRNLGKVGSKCCKHPEAKRMPCAEDYLSVVLNQLCVLHEKTPVSDRVTKCCTESLVNRRPCFSALEVDETYVPKEFNAETFTFHADICTLSEKERQIKKQTALVELVKHKPKATKEQLKAVMDDFAAFVEKCCKADDKETCFAEEGKKLVAASQAALGL

SEQ ID NO: 5 - protein, 16 aa, Artificial Sequence
MPLLLLLPLLWAGALA